European Patent Specification EP 4 308 720 B1, published May 7, 2025. Title: METHODS FOR THE SELECTIVE ANALYSIS OF CELLS OR ORGANELLES. Applicant: PARIS SCIENCES ET LETTRES - QUARTIER LATIN ECOLE SUPERIEURE DE PHYSIQUE ET DE CHIMIE INDUSTRIELLES DE LA VILLE DE PARIS Centre national de la recherche scientifique. The sequence listing filed with the application follows.

SEQUENCE LISTING (115 sequences)

SEQ ID NO: 1 - DNA, 11 bp, Artificial Sequence
  trigger oligonucleotide
cattcagttag

SEQ ID NO: 2 - DNA, 20 bp, Artificial Sequence
  amplification oligonucleotide
ctaactgaatgctaactgaa

SEQ ID NO: 3 - DNA, 13 bp, Artificial Sequence
  leak absorption oligonucleotide
aactaactgaatg

SEQ ID NO: 4 - DNA, 26 bp, Artificial Sequence
  reporting probe
catcgatatactaactgaatgcgatg

SEQ ID NO: 5 - DNA, 37 bp, Artificial Sequence
  conversion oligonucleotide
tgctaactgaagtttgactcattgctaggaccggctt

SEQ ID NO: 6 - DNA, 22 bp, Artificial Sequence
  activator oligonucleotide
gctttaaggccggtcctagcaa

SEQ ID NO: 7 - DNA, 43 bp, Artificial Sequence
  conversion oligonucleotide
tgctaactgaagtttgactcaaactatacaacctactacctca

SEQ ID NO: 8 - DNA, 104 bp, Artificial Sequence
  aptamer coupled to an activator oligonucleotide
aaggagcagcgtggaggataaacaccgtggaggatagttcggtggctgttcagggtctcctcccggtgttagggtgtgtcgtcgtggtaagccggtcctagcaa

SEQ ID NO: 9 - DNA, 99 bp, Artificial Sequence
  aptamer coupled to an activator oligonucleotide
aaggagcagcgtggaggatataggcagtggtttgacgtccgcatgttgggaatagccacgcctttagggtgtgtcgtcgtggtaagccggtcctagcaa

SEQ ID NO: 10 - DNA, 32 bp, Artificial Sequence
  activator oligonucleotide
tttttttttttgaggtagtaggttgtatagtt

SEQ ID NO: 11 - DNA, 12 bp, Artificial Sequence
  trigger oligonucleotide
cattctggactg

SEQ ID NO: 12 - DNA, 22 bp, Artificial Sequence
  amplification oligonucleotide
cagtccagaatgcagtccagaa

SEQ ID NO: 13 - DNA, 17 bp, Artificial Sequence
  leak absorption oligonucleotide
tttttcagtccagaatg

SEQ ID NO: 14 - DNA, 21 bp, Artificial Sequence
  reporting probe
attctgaatgcagtccagaat

SEQ ID NO: 15 - DNA, 38 bp, Artificial Sequence
  conversion oligonucleotide
tgcagtccagaagtttgactcattgctaggaccggctt

SEQ ID NO: 16 - DNA, 90 bp, Artificial Sequence
  aptamer
aaggagcagcgtggaggataaacaccgtggaggatagttcggtggctgttcagggtctcctcccggtgttagggtgtgtcgtcgtggtaa

SEQ ID NO: 17 - DNA, 85 bp, Artificial Sequence
  aptamer
aaggagcagcgtggaggatataggcagtggtttgacgtccgcatgttgggaatagccacgcctttagggtgtgtcgtcgtggtaa

SEQ ID NO: 18 - DNA, 14 bp, Artificial Sequence
  activator oligonucleotide
gccggtcctagcaa

SEQ ID NO: 19 - DNA, 23 bp, Artificial Sequence
  oligoucleotide
cgatcctgaatgcgatcctgaat

SEQ ID NO: 20 - DNA, 11 bp, Artificial Sequence
  trigger oligonucleotide
attcaggatcg

SEQ ID NO: 21 - DNA, 12 bp, Artificial Sequence
  trigger oligonucleotide
cattcaggatcg

SEQ ID NO: 22 - DNA, 44 bp, Artificial Sequence
  activator
ttgctaggaccggccttaaagcttttttttttttcttcaagtag

SEQ ID NO: 23 - DNA, 34 bp, Artificial Sequence
  first part cT
ttgctaggaccggccttaaagctttttttttttt

SEQ ID NO: 24 - DNA, 22 bp, Artificial Sequence
  common oligonucleotide
ttgctaggaccggccttaaagc

SEQ ID NO: 25 - DNA, 12 bp, Artificial Sequence
  flexible linker
tttttttttttt

SEQ ID NO: 26 - DNA, 20 bp, Artificial Sequence
  aT
ctaactgaatgctaactgaa

SEQ ID NO: 27 - DNA, 26 bp, Artificial Sequence
  rT
catcgatatactaactgaatgcgatg

SEQ ID NO: 28 - DNA, 14 bp, Artificial Sequence
  pT
aaactaactgaatg

SEQ ID NO: 29 - DNA, 30 bp, Artificial Sequence
  linker
cccacaggcacgctcaacgctaaccaaacc

SEQ ID NO: 30 - DNA, 52 bp, Artificial Sequence
  activator
ggtttggttagcgttgagcgtgcctgtgggttttttttttttcttcaagtag

SEQ ID NO: 31 - DNA, 42 bp, Artificial Sequence
  first part cT
ggtttggttagcgttgagcgtgcctgtgggtttttttttttt

SEQ ID NO: 32 - DNA, 49 bp, Artificial Sequence
  cT
ctaactgaatgctacttgaatgttttttttttttggttggtgtggttgg

SEQ ID NO: 33 - DNA, 63 bp, Artificial Sequence
  cT
ctaactgaatgctacttgaatgttttttttttttagtccgtggtagggcaggttggggtgact

SEQ ID NO: 34 - DNA, 35 bp, Artificial Sequence
  activator
gttggtgtggttggttttttttttttttcaagtag

SEQ ID NO: 35 - DNA, 50 bp, Artificial Sequence
  activator
agtccgtggtagggcaggttggggtgactttttttttttttttcaagtag

SEQ ID NO: 36 - DNA, 50 bp, Artificial Sequence
  activator
gagtcgggagcgctagaggtgtggttcgtttttttttttttttcaagtag

SEQ ID NO: 37 - DNA, 49 bp, Artificial Sequence
  cT
ctaactgaatgctacttgaatgttttttttttttggtgttggtttgggg

SEQ ID NO: 38 - DNA, 50 bp, Artificial Sequence
  activator
agtccgtggtagggcaggttggggtgactttttttttttttatcaagtag

SEQ ID NO: 39 - DNA, 47 bp, Artificial Sequence
  cT
ctaactgaatggagagactcttttttttttttggttggtgtggttgg

SEQ ID NO: 40 - DNA, 52 bp, Artificial Sequence
  activator
agtccgtggtagggcaggttggggtgactttttttttttttttgagtctctc

SEQ ID NO: 41 - DNA, 47 bp, Artificial Sequence
  cT
ctaactgaatggattgactcttttttttttttggttggtgtggttgg

SEQ ID NO: 42 - DNA, 52 bp, Artificial Sequence
  activator
agtccgtggtagggcaggttggggtgactttttttttttttttgagtcaatc

SEQ ID NO: 43 - DNA, 50 bp, Artificial Sequence; identical to SEQ ID NO: 38
  activator

SEQ ID NO: 44 - DNA, 50 bp, Artificial Sequence; identical to SEQ ID NO: 35
  activator

SEQ ID NO: 45 - DNA, 36 bp, Artificial Sequence
  activator
ggttggtgtggttggttttttttttttttcaagtag

SEQ ID NO: 46 - DNA, 44 bp, Artificial Sequence
  sT
tgcagtccagaagaatgactcacattgcttcattttgaagcaat

SEQ ID NO: 47 - DNA, 44 bp, Artificial Sequence
  sT
tgcagtccagaaaaatgactcacattgcttcattttgaagcaat

SEQ ID NO: 48 - DNA, 44 bp, Artificial Sequence
  sT
tgcagtccagaaatatgactcacattgcttcattttgaagcaat

SEQ ID NO: 49 - DNA, 44 bp, Artificial Sequence
  sT
tgcagtccagaaagatgactcacattgcttcattttgaagcaat

SEQ ID NO: 50 - DNA, 44 bp, Artificial Sequence
  sT
tgcagtccagaaacatgactcacattgcttcattttgaagcaat

SEQ ID NO: 51 - DNA, 44 bp, Artificial Sequence
  sT
tgcagtccagaataatgactcacattgcttcattttgaagcaat

SEQ ID NO: 52 - DNA, 44 bp, Artificial Sequence
  sT
tgcagtccagaattatgactcacattgcttcattttgaagcaat

SEQ ID NO: 53 - DNA, 44 bp, Artificial Sequence
  sT
tgcagtccagaatgatgactcacattgcttcattttgaagcaat

SEQ ID NO: 54 - DNA, 44 bp, Artificial Sequence
  sT
tgcagtccagaatcatgactcacattgcttcattttgaagcaat

SEQ ID NO: 55 - DNA, 44 bp, Artificial Sequence
  sT
tgcagtccagaagtatgactcacattgcttcattttgaagcaat

SEQ ID NO: 56 - DNA, 44 bp, Artificial Sequence
  sT
tgcagtccagaaggatgactcacattgcttcattttgaagcaat

SEQ ID NO: 57 - DNA, 44 bp, Artificial Sequence
  sT
tgcagtccagaagcatgactcacattgcttcattttgaagcaat

SEQ ID NO: 58 - DNA, 44 bp, Artificial Sequence
  sT
tgcagtccagaacaatgactcacattgcttcattttgaagcaat

SEQ ID NO: 59 - DNA, 44 bp, Artificial Sequence
  sT
tgcagtccagaactatgactcacattgcttcattttgaagcaat

SEQ ID NO: 60 - DNA, 44 bp, Artificial Sequence
  sT
tgcagtccagaacgatgactcacattgcttcattttgaagcaat

SEQ ID NO: 61 - DNA, 44 bp, Artificial Sequence
  sT
tgcagtccagaaccatgactcacattgcttcattttgaagcaat

SEQ ID NO: 62 - DNA, 44 bp, Artificial Sequence
  sT
tgcagtccagaagaaagactcacattgcttcattttgaagcaat

SEQ ID NO: 63 - DNA, 44 bp, Artificial Sequence
  sT
tgcagtccagaagaaggactcacattgcttcattttgaagcaat

SEQ ID NO: 64 - DNA, 44 bp, Artificial Sequence
  sT
tgcagtccagaagaacgactcacattgcttcattttgaagcaat

SEQ ID NO: 65 - DNA, 44 bp, Artificial Sequence
  sT
tgcagtccagaagatagactcacattgcttcattttgaagcaat

SEQ ID NO: 66 - DNA, 44 bp, Artificial Sequence
  sT
tgcagtccagaagattgactcacattgcttcattttgaagcaat

SEQ ID NO: 67 - DNA, 44 bp, Artificial Sequence
  sT
tgcagtccagaagatggactcacattgcttcattttgaagcaat

SEQ ID NO: 68 - DNA, 44 bp, Artificial Sequence
  sT
tgcagtccagaagatcgactcacattgcttcattttgaagcaat

SEQ ID NO: 69 - DNA, 44 bp, Artificial Sequence
  sT
tgcagtccagaagagagactcacattgcttcattttgaagcaat

SEQ ID NO: 70 - DNA, 44 bp, Artificial Sequence
  sT
tgcagtccagaagagtgactcacattgcttcattttgaagcaat

SEQ ID NO: 71 - DNA, 44 bp, Artificial Sequence
  sT
tgcagtccagaagagggactcacattgcttcattttgaagcaat

SEQ ID NO: 72 - DNA, 44 bp, Artificial Sequence
  sT
tgcagtccagaagagcgactcacattgcttcattttgaagcaat

SEQ ID NO: 73 - DNA, 44 bp, Artificial Sequence
  sT
tgcagtccagaagacagactcacattgcttcattttgaagcaat

SEQ ID NO: 74 - DNA, 44 bp, Artificial Sequence
  sT
tgcagtccagaagactgactcacattgcttcattttgaagcaat

SEQ ID NO: 75 - DNA, 44 bp, Artificial Sequence
  sT
tgcagtccagaagacggactcacattgcttcattttgaagcaat

SEQ ID NO: 76 - DNA, 44 bp, Artificial Sequence
  sT
tgcagtccagaagaccgactcacattgcttcattttgaagcaat

SEQ ID NO: 77 - DNA, 44 bp, Artificial Sequence
  sT
tgcagtccagaagaatgactcaaattgcttcattttgaagcaat

SEQ ID NO: 78 - DNA, 44 bp, Artificial Sequence
  sT
tgcagtccagaagaatgactcatattgcttcattttgaagcaat

SEQ ID NO: 79 - DNA, 44 bp, Artificial Sequence
  sT
tgcagtccagaagaatgactcagattgcttcattttgaagcaat

SEQ ID NO: 80 - DNA, 44 bp, Artificial Sequence
  sT
tgcagtccagaagaatgactctaattgcttcattttgaagcaat

SEQ ID NO: 81 - DNA, 44 bp, Artificial Sequence
  sT
tgcagtccagaagaatgactcttattgcttcattttgaagcaat

SEQ ID NO: 82 - DNA, 44 bp, Artificial Sequence
  sT
tgcagtccagaagaatgactctgattgcttcattttgaagcaat

SEQ ID NO: 83 - DNA, 44 bp, Artificial Sequence
  sT
tgcagtccagaagaatgactctcattgcttcattttgaagcaat

SEQ ID NO: 84 - DNA, 44 bp, Artificial Sequence
  sT
tgcagtccagaagaatgactcgaattgcttcattttgaagcaat

SEQ ID NO: 85 - DNA, 44 bp, Artificial Sequence
  sT
tgcagtccagaagaatgactcgtattgcttcattttgaagcaat

SEQ ID NO: 86 - DNA, 44 bp, Artificial Sequence
  sT
tgcagtccagaagaatgactcggattgcttcattttgaagcaat

SEQ ID NO: 87 - DNA, 44 bp, Artificial Sequence
  sT
tgcagtccagaagaatgactcgcattgcttcattttgaagcaat

SEQ ID NO: 88 - DNA, 44 bp, Artificial Sequence
  sT
tgcagtccagaagaatgactccaattgcttcattttgaagcaat

SEQ ID NO: 89 - DNA, 44 bp, Artificial Sequence
  sT
tgcagtccagaagaatgactcctattgcttcattttgaagcaat

SEQ ID NO: 90 - DNA, 44 bp, Artificial Sequence
  sT
tgcagtccagaagaatgactccgattgcttcattttgaagcaat

SEQ ID NO: 91 - DNA, 44 bp, Artificial Sequence
  sT
tgcagtccagaagaatgactcccattgcttcattttgaagcaat

SEQ ID NO: 92 - DNA, 44 bp, Artificial Sequence
  sT
tgcagtccagaaggttgactcacattgcttcattttgaagcaat

SEQ ID NO: 93 - DNA, 44 bp, Artificial Sequence
  sT
tgcagtccagaaggaagactcacattgcttcattttgaagcaat

SEQ ID NO: 94 - DNA, 44 bp, Artificial Sequence
  sT
tgcagtccagaagggagactctcattgcttcattttgaagcaat

SEQ ID NO: 95 - DNA, 44 bp, Artificial Sequence
  sT
tgcagtccagaacggagactctcattgcttcattttgaagcaat

SEQ ID NO: 96 - DNA, 44 bp, Artificial Sequence
  sT
tgcagtccagaagggagactcttattgcttcattttgaagcaat

SEQ ID NO: 97 - DNA, 44 bp, Artificial Sequence
  sT
tgcagtccagaagcgagactctcattgcttcattttgaagcaat

SEQ ID NO: 98 - DNA, 44 bp, Artificial Sequence
  sT
tgcagtccagaagggagactctgattgcttcattttgaagcaat

SEQ ID NO: 99 - DNA, 44 bp, Artificial Sequence; identical to SEQ ID NO: 46
  sT

SEQ ID NO: 100 - DNA, 50 bp, Artificial Sequence
  sT
tgcagtccagaagtttgactcacattgcttcattttgaagcaatgtgagt

SEQ ID NO: 101 - DNA, 35 bp, Artificial Sequence
  first part sT
tgcagtccagaagtttgactcacattgcttcattt

SEQ ID NO: 102 - DNA, 17 bp, Artificial Sequence
  second part sT
tttgaagcaatgtgagt

SEQ ID NO: 103 - DNA, 43 bp, Artificial Sequence
  sT
tgctaactgaagagtgactcacattgcttcattttgaagcaat

SEQ ID NO: 104 - DNA, 43 bp, Artificial Sequence
  sT
tgctaactgaagagagactcacattgcttcattttgaagcaat

SEQ ID NO: 105 - DNA, 43 bp, Artificial Sequence
  sT
tgctaactgaagagcgactcacattgcttcattttgaagcaat

SEQ ID NO: 106 - DNA, 43 bp, Artificial Sequence
  sT
tgctaactgaagattgactcacattgcttcattttgaagcaat

SEQ ID NO: 107 - DNA, 43 bp, Artificial Sequence
  sT
tgctaactgaatcatgactcacattgcttcattttgaagcaat

SEQ ID NO: 108 - DNA, 49 bp, Artificial Sequence
  second part of sT
tgctaactgaagtttgactcacattgcttcattttgaagcaatgtgagt

SEQ ID NO: 109 - DNA, 43 bp, Artificial Sequence; identical to SEQ ID NO: 104
  second part of sT

SEQ ID NO: 110 - DNA, 43 bp, Artificial Sequence; identical to SEQ ID NO: 104
  second part sT

SEQ ID NO: 111 - DNA, 44 bp, Artificial Sequence
  cT
tgctaactgaagagagactcacttgctaggaccggccttaaagc

SEQ ID NO: 112 - DNA, 44 bp, Artificial Sequence; identical to SEQ ID NO: 111
  cT

SEQ ID NO: 113 - DNA, 24 bp, Artificial Sequence
  cT
gtggtctgagtttgactctaactg

SEQ ID NO: 114 - DNA, 22 bp, Artificial Sequence
  second part cT
ctaactgaatgctacttgaatg

SEQ ID NO: 115 - DNA, 22 bp, Artificial Sequence
  second part cT
ctaactgaatgctacttgaatg